European Patent Application EP 4 141 123 A1, published March 1, 2023. Title: Haploid Inducer. Applicant: KWS SAAT SE. The sequence listing filed with the application follows.

SEQUENCE LISTING (24 sequences)

SEQ ID NO: 1 - protein, 15 aa, Artificial Sequence
  amino acid consensus sequence of the N-terminal tail domain of the CENH3 (part A)
  misc_feature (7)..(8): Xaa can be any naturally occurring amino acid
MARTKHXXARRSRKR

SEQ ID NO: 2 - protein, 14 aa, Artificial Sequence
  amino acid consensus sequence of the N-terminal tail domain of the CENH3 (part B)
  misc_feature (6)..(6): Xaa can be any naturally occurring amino acid
QSQTQXKKKHRYRP

SEQ ID NO: 3 - protein, 15 aa, Artificial Sequence
  amino acid consensus sequence of the Alpha-N-helix of the CENH3
  misc_feature (10)..(10): Xaa can be any naturally occurring amino acid
GTVALREIRXFQKTT

SEQ ID NO: 4 - protein, 11 aa, Artificial Sequence
  amino acid consensus sequence of the Alpha-1-helix of the CENH3
AAPFIRLVREI

SEQ ID NO: 5 - protein, 13 aa, Artificial Sequence
  amino acid consensus sequence of the loop1 of the CENH3
  misc_feature (7)..(7): Xaa can be any naturally occurring amino acid
TNFLAPXEVTRWT

SEQ ID NO: 6 - protein, 29 aa, Artificial Sequence
  amino acid consensus sequence of the Alpha-2-helix of the CENH3
AEALLALQEAAEDFLVHLFEDAMLCAIHA

SEQ ID NO: 7 - protein, 7 aa, Artificial Sequence
  amino acid consensus sequence of the loop2 of the CENH3
KRVTLMK

SEQ ID NO: 8 - protein, 10 aa, Artificial Sequence
  amino acid consensus sequence of the Alpha-3-helix of the CENH3
KDFELARRLG

SEQ ID NO: 9 - protein, 6 aa, Artificial Sequence
  amino acid consensus sequence of the C-terminal domain of the CENH3
GKGRPW

SEQ ID NO: 10 - DNA, 537 bp, Artificial Sequence
  Arabidopsis thaliana - cDNA coding for CENH3
atggcgagaaccaagcatcgcgttaccaggtcacaacctcggaatcaaactgatgccgccggtgcttcatcttctcaggcggcaggtccaactacgaccccgacaaggagaggcggtgaaggtggagataatactcaacaaacaaatcctacaacttcaccagctactggtacaaggagaggggctaagagatccagacaggctatgccacgaggctcacagaagaagtcttatcgatacaggccaggaaccgttgctctaaaagagattcgccatttccagaagcagacaaaccttcttattccggctgccagtttcataagagaagtgagaagtataacccatatgttggcccctccccaaatcaatcgttggacagctgaagctcttgttgctcttcaagaggcggcagaagattacttggttggtttgttctcagattcaatgctctgtgctatccatgcaagacgtgttactctaatgagaaaagactttgaacttgcacgccggcttggaggaaaaggcagaccatggtga

SEQ ID NO: 11 - protein, 178 aa, Arabidopsis thaliana
MARTKHRVTRSQPRNQTDAAGASSSQAAGPTTTPTRRGGEGGDNTQQTNPTTSPATGTRRGAKRSRQAMPRGSQKKSYRYRPGTVALKEIRHFQKQTNLLIPAASFIREVRSITHMLAPPQINRWTAEALVALQEAAEDYLVGLFSDSMLCAIHARRVTLMRKDFELARRLGGKGRPW

SEQ ID NO: 12 - DNA, 4001 bp, Brassica napus
  Intron (1892)..(1972)
  Intron (2020)..(2104)
  Intron (2148)..(2208)
  Intron (2264)..(2358)
  Intron (2399)..(2507)
  Intron (2624)..(2755)
  Intron (2832)..(2933)
  Intron (3012)..(3091)
tgtccgggaggatccaccggcggtggtcgttactccattttaacttgatgtcttgaaagcagaggacatggtatggtggcggcagaatctatttttagttgttaatttttcttttcctctgattctttttatttttttcgaatgaactaactttgggtttattcagaagaattatcatctaaaaactgattcaataaacaaaataatttacatatttcacaatgagccattagtaaacaagtcgaaagtgaaaccaaatgggaagagaacaattttaataaaaatatgttctaatttcctactttttatgaattgaactcccgaagagaatggccgaagaacggagtaaaagctcaatgattgtaaaagctatgtattctcttgctttgaggaaaaagctttttgtttgcactcataggcctgatatgttgtgatggctctttacatattgggtcttttgtggtctattaaacggttactgaagaattagtttatcgcatttaaaaaaaaatatttgaaaaccacatatctaaaatctcaatatattatttattgatagatgaaaagaaaaatagtttataaaataatattaattggtaaatggaagtcaaaattttacatttaatacatgactagttcgattctccggctgaaacccatttaccactgagccaagaccacttgattatatatatcaagctcttgttttttgcattaacaaaagttgcatccaaaatttcaaaacaacaactaaattaatgtctttctattttcaaagttttatctccaaacctattaatagtttaatttttttttttaaaattaggaaaccggttaaaatatattttaaatacaaaaaacttaaacaatgaatcatttatttatttattcttcaaaatttaaatatccgaacccggcccaaaatatccgaacccgaacataaaatatccgaacccgactcgaagtgtagaaaatatccgaacgggttttatacctttatactgaaataccctatacgaacccgaatgtgtatccgaacgccccctacaatatatgatcatcatttgtatcttgattgaacaaaaaaaaagttaaactattgatcacaaaattttcaatgtgagacttttaccatttttagtcatttatagtcgtttttaaaaattcaaaatataacttataagaaaaaatctaattttttttattatatgcttaatgtgattgtttaatttcttttaataatataaaattaaacaaaaaatgagaggttaaaaaaattgttatcaaatatgtattattcataatcattaattgtcatatatatgttaattatattaggtaatttcgtagtttttatttaagaaaagaaaaaaatattattttgtacactactaattaatttgatagttagtttaataaaaaatatattatattattatatggaccaacttatttttctaaaaaaaaaccactgttttaaaaaccaaaccaactataaaccggagatataccggattgagtggctaaaacactctttgtatatatgtgctgagcaaaccctctgagtgagatggcgtgttaagaagtaggaggaccattcatgcctcttatgagttgtagtctgtgtgtacaaaaaagaagcgttggtgtgaaagaaagcagaaggatttgaaaatcaaaaaaattgaaggagaagcgggaaaacaaataatctctccctccgcttttttttctccaaataatcaatctctcatttcatttgttaacccaagtttttgataattatttcaaaggggtttatttatcttttattcctccggcggcagtaagtagtaatcaatggcgagaaccaaacatttcgcttccagggcacgagatcgcaatcgaactagttagtactctctctctctctgccttttttttgatatttattttctaggttaaaccctaatttggcatctgaaatttgtagatgcgactgcttcatcttcggcggcggcggcggaaggtccgagtgcggtacgtcatctattttcttttcccgttttaggtttttacgcaaatctcgttactgtttttttgacgaatcgattgaaatgtgtagaccccgacgagaagagaaggcagccaaggagaagctcaacagagtgagtctttctatttcattttctgagatccatgaatccttttcatctctcgtgtgttgtgacatgaatcaattgcagcagcaactcctactacgactccaccagccggtagaaaagtaagttacatttccatttcacaccattcatttgcttctttatcaacaaactgctctctcatctgttttttttgttttgttttggttttgtgaagaaaggagggactaagcgaactaaacaagctatgcctaaaagttagtgacagattttaaaatctctattttggatcatcattctctcaggacatgtctatttgcatttgttcttattatgtctgtctgtctgtctttgtcccccttgtaggttccaacaagaagaagacattccgttacaagcctggaaccgttgccctcagagagattcgccatttccagaagaccaccaaacttcttatccctgccgctagtttcatccgagaagttagtaatgaactttgttattcatacattcccgcttacttgttttcaatgactctgcaattactgatatagaatttggagcaaccattatggggtgatttctctaactacaaattactaatactatcccaggtgagaagtgtcacccagatctttgcccctcccgatgttacccgttggactgctgaagctcttatggctattcaagaggtacgtgtactccttccctcttttgtttcctattttccacttgatgtctaatttaaactgatcgttttttttttatatttcttttggtgtggggcggggcaggcggctgaagattttttaattggcttgttctctgatgctatgctttgcgctatccatgcaaggcgtgttactctaagtaagtagtactccccaaaataaggaaacccattttatatacaacattgcctcatccatgtctgcttctcttcatatcagtgagaaaagattttgagcttgcacgccgtcttggaggaaaaggcagaccattgtgatcgtttcgcaggttgtataactttgttcactccttatgtcttgtcatttgtgatctgactgacactttcttttgaaacataactgcttgattcaatatctaggctgtaaaacttatccctccttgtttactatcttatatgctttttccttggaattgatagtttccattgagatttcacttgcacgaaacatatctgctttctcaatatctctcagtcttagaaagggctattgactaaaagaaaagaaaatttagaggaagatttgtaaagacatgtgtttagagagggcttaattaaaaacacacgcttctgctagccttgctatttgattcccaatttcaacttttttcgaggcatattataaagtttttaaatgtacttggcacttcaacttttataatttatataacgattttattctaatagagcatttgtgatttcatagtgttgtcatgaaactcaagtaattcacaccgtccgatgttgctattgtctaataaaatgttgaaaaaattgtcaaaacagaacaaaaaacaacatagttgtctctatggtataaaactatcactaagttgtctctatagtataatatttttcgcaatcccaaaactaatttttctttaatcaaattaaacataaactaaaaccatttttaaaaagtttaatggaaaaagataaaaaaataaggtaatctcgtaatgttttaaaaaggaaaaaaaatgtaaaaacaatttaaaaaaaagaacacacgacacagatcaaaaatatcatgtaatctaattgcatttggtttctaaaatcttccaaaactattcttttaaaattctctaaggtaaaacttgattccaata

SEQ ID NO: 13 - DNA, 540 bp, Artificial Sequence
  Brassica napus - cDNA coding for CENH3
atggcgagaaccaaacatttcgcttccagggcacgagatcgcaatcgaactaatgcgactgcttcatcttcggcggcggcggcggaaggtccgagtgcgaccccgacgagaagagaaggcagccaaggagaagctcaacagacaactcctactacgactccaccagccggtagaaaaaaaggagggactaagcgaactaaacaagctatgcctaaaagttccaacaagaagaagacattccgttacaagcctggaaccgttgccctcagagagattcgccatttccagaagaccaccaaacttcttatccctgccgctagtttcatccgagaagtgagaagtgtcacccagatctttgcccctcccgatgttacccgttggactgctgaagctcttatggctattcaagaggcggctgaagattttttaattggcttgttctctgatgctatgctttgcgctatccatgcaaggcgtgttactctaatgagaaaagattttgagcttgcacgccgtcttggaggaaaaggcagaccattg

SEQ ID NO: 14 - protein, 180 aa, Brassica napus
MARTKHFASRARDRNRTNATASSSAAAAEGPSATPTRREGSQGEAQQTTPTTTPPAGRKKGGTKRTKQAMPKSSNKKKTFRYKPGTVALREIRHFQKTTKLLIPAASFIREVRSVTQIFAPPDVTRWTAEALMAIQEAAEDFLIGLFSDAMLCAIHARRVTLMRKDFELARRLGGKGRPL

SEQ ID NO: 15 - DNA, 3088 bp, Sorghum bicolor
  Intron (377)..(487)
  Intron (514)..(618)
  Intron (662)..(1094)
  Intron (1217)..(1312)
  Intron (1391)..(2087)
  Intron (2164)..(2556)
catctctcactgccatccgggtccactactcccaacgttcggcacgccaggtatagccgttaccccggtaggccccactggtacacggacaaaggttagcggtcaccgcgaatcgtgaatacttgtgactacggggtgctaattataaaaacgccgcacatcctttcgtttcgccatttcaccccccttcccttcccgtagagaggaaaaaaacccaccgtcgacccgcccggccgcccgagagttctgaatcgaaaccgtcggccgcgaccgcgagagcagcgcggggcgcccaccgtgatggctcgaaccaagcaccaggccgtgaggaagctgccgcagaagcccaagaagaagctccagttcgagcgcgcaggtaagcccgcgtccccgcgctgaacccccctccgcctcgcgagcagacgctgccgctgctctccgtcgcccctggtgctaagcgcgttccttttttttccttcttttgcaggtggggcgagtacgtcggcgaccccggtgagtgcgtgcgtgcgtgcgggaattggttttagccctccttttgcggtttcgccttttgttgggctggtctcacttgcttgcaatctgtttgatggaatgcaggagaggaggaatgctgggaccgggggaggagccgcggctcgcggtgaggatctctttgtcgttgctgggtttgggaatttccggcgcgaaattatgtggatttctaggtttatctgccgtctttcttcttgtcttctcttttggctctggggtgagaagttagggtggttgggcggacatggtgcgttatttcgccgtatcgtttggtttggtgctttctcatccttttaattccaacatgccttgtaaaaattgcacaagatttgttttttcatgcatgtctcagtgttgctaatttgcttttccggttcggttggtagaattcaatttcttggcgcaatatgcatcttcttttgttgcaacatgagggcgaatgtgccagttccatatgggcgtcgcggttttgaagttactaccttgcttgctcttcgtattataggcgtcattcacaatagtatgttttcttggagatgcagttgcacgggggcgtgtggagaagaagcatcgctggcgggcagggactgtagcgctgcgggagatcaggaagtaccagaagtccactgagccgctcatcccctttgcgcccttcgtacgtgtggtgggtgcatcttgtaccaattgttgtccactccatagaatgggtttgttctgcagtctgtctgatggaaagttattcttctgagaaaaaatgcaggtcaaagagttaactgcattcataacagactggaggatagggcgctacacccctgaagccctccttgcgctgcaagaggtcagttatgaaacatgtcttgtgtatcagttaagatcatcttctatagacataattgttatcatgaagtctttttctgttaatcggtctggtactacttaataatcaggatttcagattgctgcctttcctagtggtgtagtcaaaagggaatttaagtgctgttaggtactgtttgttttggtgttttgaaccctgccgcgatcggttgttgttattccatgtttgtttctgtggcagcggacgttcacggtgagatgggatacgggcgtgtgaaacatagttacggtccatcttcatggcttatccatttacgctgctcgtccgctcacttgttatgtgcggcaaccaaacttttgttactagtgtaactggtagcgttgcaaatctttccatttgcgttaccactccctatgggagccaaacagcaccttagtgtagattccatttgtattacttgagctagcttccttgctattggtgcctcgattgtactgttatgatcgaagtgctgaaaactttgtcgcctgcatagcatgattagagaacttgagtttacatttattcaataccttaagactgcatttcgtatagataaattatttttcctaattgttctggttaactgttttaggtttccatatttttgtatgtgtatcatttaaattattgtgttgtttttcctccctgtctacaggcagcagaattccacttgatagaactgtttgaagtggcgaatctgtgtgccatccatgccaagcgcgtaacagtcagtaagttatcactgaatgaactccttttcctctgtactattacgcctaatggagatgtgtgatgcatttttggttacacgattctttagtgattctgcttcagttggatatgataaatctagatgttatttaaagtggcaaattgcttacgagtggaaatagtaatgttcaaatagtgaaaagtgcaattaaacttttaataggccattatatggtttgattgtcaacaaatgcatcaagaaatagtaaatattataacagttatggcttagagagtggacaaaaaatcggtaatggtgagctttgtataaacactaaaactggctgagaaatctgataactcaaggatctataggaaatgtattatcctaaatgttttccttcctgctgcagtgcaaaaggacatacaacttgcaaggcgtatcggaggaaggcgttggtcgtgatatccattctgattctgattaccttgttcgggtggaatttgtttagaggagttagacattagtcttgttgaatgctgtgcatggttcctaatctgtttcacagttagtgggctcttctgggatgatctgttaacacctgtggagtatgttatgtaggaaacacctgaactgaacaacccaaagttgttttggttgctcttcaaccatttgtttgcttcagagatcgattctaaactgcatgctaattagtctatggttgaacaaaaattatcaaatataaatgaaagtgatatagtagcaaaatccaaaaaaaaaaggatccaaacaaggcctaaaatcatggttctttctccttttgaactgggtgcaagtatggacaggcacagaagaaaaccgcctagcaaaccgtttgtttttttttcttcgttgtaccacacgacactgttcgttcctagttgcgcctttttgttgtagaagtc

SEQ ID NO: 16 - DNA, 471 bp, Artificial Sequence
  Sorghum bicolor - cDNA coding for CENH3
atggctcgaaccaagcaccaggccgtgaggaagctgccgcagaagcccaagaagaagctccagttcgagcgcgcaggtggggcgagtacgtcggcgaccccggagaggaggaatgctgggaccgggggaggagccgcggctcgcgttgcacgggggcgtgtggagaagaagcatcgctggcgggcagggactgtagcgctgcgggagatcaggaagtaccagaagtccactgagccgctcatcccctttgcgcccttcgtacgtgtggtcaaagagttaactgcattcataacagactggaggatagggcgctacacccctgaagccctccttgcgctgcaagaggcagcagaattccacttgatagaactgtttgaagtggcgaatctgtgtgccatccatgccaagcgcgtaacagtcatgcaaaaggacatacaacttgcaaggcgtatcggaggaaggcgttggtcg

SEQ ID NO: 17 - protein, 157 aa, Sorghum bicolor
MARTKHQAVRKLPQKPKKKLQFERAGGASTSATPERRNAGTGGGAAARVARGRVEKKHRWRAGTVALREIRKYQKSTEPLIPFAPFVRVVKELTAFITDWRIGRYTPEALLALQEAAEFHLIELFEVANLCAIHAKRVTVMQKDIQLARRIGGRRWS

SEQ ID NO: 18 - DNA, 5834 bp, Zea mays
  Intron (1820 )..(1917)
  Intron (1944 )..(2035)
  Intron (2085 )..(2239)
  Intron (2356 )..(2446)
  Intron (2525 )..(4530)
  Intron (4607 )..(5346)
ttatgtagaggcaattgcagtagtgcctctgttttagagtgtaactacagatttgtccctatttttttagagtttgcgtgtttgtccctgttttttcaaatcaaactattgtatacccctactccattagttatacttaacaatgttaagtcttgataaaaagacaagggataattggattagtgaccctgttttagagtgtaattatagctttgcccgatgttttagacttcacatgtttttatgacaattcaaattgtttccataacatcttaaattattttgacaacatttagaattgttttgcaataatttaaattatttccaaaataaaaatattttgacaattattttatcaacaaattaaattattttttttacaaaataatttgtcaaggtacttttttaaaattttgaaaataatcaaattattgtaaatataatttgaattgttgcgaaaataatttggattgtcataaaaacacgtaagtctaaaaattaggcgtaaaactacaattatactctaaaaaggtggtaatggcgtagttgttccttgtctattttatcaagacatagcaccgtgcagtacaactaatggagtagtgacatacaacaattttgttttaaataataggggtaaatacgcaaagtctaaaaaacagaggtaaatctacaattacatgttaaaatagaggcatcgatacaattgtaccttttatatagcagcatgcgccctgttgggatacaattgtacctttcacatgtcttctagatggttcccaaccctttggccaagatcgtacagataatattgcgaggagcccaaatcaacggtgtccatatgttatgttgatgtggatggtttacctaggcgcaaaagtgcgctggtttcgtccgtacaaatatactttaagtatggttttgatttttttctatttttcattttttaaataaaacgagacaatcaaatctgatataaaaatcaaatgaattataaatagagacggaaagagtatatatatttgttttgctattatttaaagtattaaaagatagtggacgaatgaacgtcctctatgtttaaaagaacgttttagaggacgttgtgttgttgaaggaaatatgaaaaaaaaatcttctgcatatttagaagggaggagcgtttacacattactttcgggacttcaacccaaatatgtcaaggtttgtgagtggctcagtgcggaaaaaaaatcctatatataccagatgtaaacactatcttttacagcctatcacattcacatttagaggttcacaaagatagatcaaaatttataaaataatcatttaatattttttttattttatttatatggataagcagctggtgtatgtgaggagctgtaaaagatattttttacatccgagatgtaaagattttttttaactcaatgctggttaccggctgggaggacgatgataaagaaagcatctctcactgcattccgggcccactactcaaacgttcggcacgccaggttggcaggtagccgttacatcgataggcactcggccactcgcacgcagacaccacaccagtgtgctcagtgctcactgctcaccataataacgctgcacctcttttcatttcaccatctcctgcccccttaaaaaaaagactcaccgtcgacacgccctcccgtcccgagagttctgaatcgaaaccgtcggccacgagagcagtgcgaggcgcccaccgcgatggctcgaaccaagcaccaggccgtgaggaagacggcggagaagcccaagaagaagctccagttcgagcgctcaggtaacccgggtcccgcgctcccccccgcttcgcaagcagacgctgtcgcttctctccgaccctggtgctaagcacgttccttgttccgtcttttgcaggtggtgcgagtacctcggcgacgccggtgagcgcgtgcgtgcggggatcagttccctccttttgcctttttttgttgggctgctcttacttgcttgcaagctgtttgatggaatgcaggaaagggctgctgggaccgggggaagagcggcgtctggaggtgactcaggtgaggacctatttgtcgttgctggatgctgggtttcgcttgcaatctaattttgttgcaagatgagggcgaatgtgccagttccatgtgggtgtcatggtctcggagttactaccttaattgctcaccatagtatgttttcttaaaaaaaacagttaagaagacgaaaccacgccaccgctggcggccagggactgtagcgctgcgggagatcaggaagtaccagaagtccactgaaccgctcatcccctttgcgcctttcgtccgtgtggtgggtgcaggcgtgtttgtcctctgcatagtatggggttgttccgcattctgtctaatggaaagttattcttctgagaaaaaaaatgcaggtgagggagttaaccaatttcgtaacaaacgggaaagtagagcgctataccgcagaagccctccttgcgctgcaagaggtcagttatgaaaaatgtcttatctctctgttaagatcctcttcatatacatagttgctattgctatcgtgaagtcttttttttctgttaattggtctggtactacttactagtcaggatttcatattgcggtttttcctagtggtgtgtagttaaaaagtagtttaattgcttttagttaaaaggggtgttcagggctaaagatcaactatgagaaaacagaaattttcccaattcgatacccgacagcattatggcctgcgctaatggaggtgtttccgggcaaatactctagcctacctgggaagtaccttgggttgccccttcatttcaggaaagtaaaaaggaatgatcttcaacctctaatcgaaaaaatcaacaacaggctggccttgctggaaaggcaagatgttgtccaaggctggtatagaaactcttgtaaaatcgatgctatccgcacaaccaatctaccatctaatggtttttccacctcaaaaatggctgctgcaaacaattgacaaaatacgaagaaacttcctgtggagagggagcaatccagaagtttgcagcgggggtcactgcctcgtcaactggcccgtaacttgcctcccaaagaacaagggaggtcttggaattctggaccttgatcgttttgcgagggggctaagactaagatggctgtggctacgatggaagagcaaagatagggcgtggactgccttgaagcttccttgtgacaaaactgatgaagatctcttcaatgcttccacaactgtcacggtaggcaatggaaagatagctgaattctggaattctagttggatccaaggccaagcccctaagaacattgcgccaacactgttcaagaaggaaaagaggaagaacatcacggtcgccaaagcgctcactaacaacaattggattcgtttatgctcaccatacacgggtgagggggagtttagagaggtcgtctctctttggcaggccataggtaacatgcaagagcttaacggtttggaagacaacatctcttggagatggacggcagatgggcagtacagtgctagcagtgcatacaaaatccagttcgcatccaatttcactaaaatgaacctctgccctatttggaaggctaaagtggaaccgaaatgccgattttttgcttggacactacttcataagagaattctgactgccgataaccttcataaaagaggttgcaactcagcctcagaaacaattccccacttatgcaaggattgcccctttagtagagaggtgtggaacaaagttttgtctcgggccaactttcctttactgactgggtctcccagtgacacttctttgtatgattggtggacggacatgtgcagcctttgcagcagacaggcaagaagaggtttcgacggtctgctatttcacttttggtggaacttatggctggaaagaaataacagaatctttcaaaggcagcgtagaagtgtagatcaagttgctctggcagtcaaggattatgctagtagctgaagtctagttggtttggactagtggttttgttgcttttctttttaatttctttttagttctttttatgttgttttcgtttccttaagttgcttggagtctgtattatcctctttcttctaatatagatcggagcgacaaaccttttgccccttcctttcaaaaaaaagttaaaagggaatttaactgctttcctagtggtgtagttaaaatggatttcatattgcggcctttcctagcttgcttgctattgattggactatagtgatccaaatgctgataactttgtcgcttgtgtaggcatggttagagagcttagagtttgcatttattcaataccttgagactgcatttcatatacataaattattcatgattatttcttttctctatttgttctggttaattaagagttttaggtttccatatttttgtacgtgcatcatttaaattcttgtattgtttttcgttcttgtctacaggcagcagaattccacttgatagaactgtttgaaatggcgaatctgtgtgccatccatgccaagcgtgtcacaatcagtaagttatcactgagtgaactcctttttctctgtagcattactcctaatgaatatgtgtgatgcattttggttgcacgattctttagtgattctgcttcagatggatatgataaatctagatgttattttgaagtggcgaattgcttacgagcggaaatagtaatgttcaaatagcgcaaagtgcaactgttgacttttagtaggccatttatatggtttgattaccaacaaatacgtcaatcatatgatttgattatcaacaaaggaatcagctatatggtttgattatcaacaaaggaatcagctaggtttgcttatcaacattcaacaaaggcatcaagtaatactccatccgtttcaatttataattcgtttgactttttttatctaagtttgatcggctcgacttattaaaaaaaatcataattattgttaatttttgttgtgatattgtttagtataatatactttaaatgtgactttgagtttttcattttttcgcaaaaaaaaatgaataggacgagccggtcaaacgtgacacaaaaaagtcaaacgaattataatttgggacacacggagtagtaaataatgtaacaacttagagagtgggacaaaaaaatctctagtggtgctaaatttagttcagctttgtataaacacaagcattgattgagaaatctgacaactcaaggatctgtaggaaatgtgttaccctaaatgttttccttactgatgcagtgcaaaaggacatacaacttgcaaggcgtatcggaggaaggcgttgggcatgatatataatatccattctgattgcatcattcttgtgaatttgtttgtaggagctagacattagtgttgttgaatgctgcatggttcctaatccttttcgcagtctaacatctgtggagttagtatgttacatggcaacagctgaacatctgtggactatatggcaacagccgaagattgtgtctgtgggataactggttgttttggttgctcttcagtagtttgtttgcttcaggtaaccatgctgcgaactatgatgttttcattctcggtttgcttcagctaaccgagatcgattcagtctgcagtatggactatggagtaaactgcatgctgaaacccgaaccactgctgaaactgcatgctgaaacccgaaccactgctacggcagttgccaggatagcaggagggcctttatgcacagtggaattgagtag

SEQ ID NO: 19 - DNA, 471 bp, Artificial Sequence
  Zea mays - cDNA coding for CENH3
atggctcgaaccaagcaccaggccgtgaggaagacggcggagaagcccaagaagaagctccagttcgagcgctcaggtggtgcgagtacctcggcgacgccggaaagggctgctgggaccgggggaagagcggcgtctggaggtgactcagttaagaagacgaaaccacgccaccgctggcggccagggactgtagcgctgcgggagatcaggaagtaccagaagtccactgaaccgctcatcccctttgcgcctttcgtccgtgtggtgagggagttaaccaatttcgtaacaaacgggaaagtagagcgctataccgcagaagccctccttgcgctgcaagaggcagcagaattccacttgatagaactgtttgaaatggcgaatctgtgtgccatccatgccaagcgtgtcacaatcatgcaaaaggacatacaacttgcaaggcgtatcggaggaaggcgttgggca

SEQ ID NO: 20 - protein, 157 aa, Zea mays
MARTKHQAVRKTAEKPKKKLQFERSGGASTSATPERAAGTGGRAASGGDSVKKTKPRHRWRPGTVALREIRKYQKSTEPLIPFAPFVRVVRELTNFVTNGKVERYTAEALLALQEAAEFHLIELFEMANLCAIHAKRVTIMQKDIQLARRIGGRRWA

SEQ ID NO: 21 - DNA, 8441 bp, Beta vulgaris
  Intron (99 )..(203)
  Intron (245 )..(331)
  Intron (344)..(488)
  Intron (591)..(3263)
  Intron (3339)..(4377)
  Intron (4458)..(8130)
ctactctttctctctctctctctctccatttctgtttgaaatcatgagagttaaacacactgctgccaggaaatcaaccaccaacggtcctcgttcaagttagtttcctctctcttcttcttttttgttcgcattctctcaatctatatttcaaatttgaaaaaaattgtgatgctcataaaccctaaaattttcttgtacagaggctcagaaatctccgcgcagtttgcaatcaccacaatcggttctctctttgtacttttgatttgtttttccttcatttgttcgatgaatggctcttaattgtcttttatttacttgaaaattgcagccttctagtagttcaaagcgcaaatcactcagaaacactgatgcaactcctcaaagtaactttttctttaatattaggtttaattttactgctgtttgccaaattctgttgaaattgtaaaatattttttttcttaaatttgacggtttcagagaagaaggcttaccgccgtaagccgggcactgtggcactctgggaaatacgcaaatttcagaagtcattcaagcccttgattcctgctgcgcctttcattcgaacagtatgtattttttttgtttgtacttaataaatgaattttggactggtgtttgtgtggctgcatagaaatatatttccatacaactgaaattgtcctaggaggtatcgatgaatgtttgctacaaaataaataaatataagtgattatatcttgttaaaaagccattataattgcaacttatatgtatgttgtaatgaggtcaactagctattttgtgcaaagtcacccacactttaacataattttgtgctctcgtaaccttaaaaaaatataagtaaagggttgatttggtctaattagagctgatgaaacccaattagattgaaacataaggtgaaatcaggtggtgatcagcttcaattagatctaataagtgcagtttagtttagcttcggtgaaatgaacacacccttaaagatagaaaatcgacactatatatggtcctttttagatatgatagttcgatattctgttttggggtgtgttgaatgattaaatggagtggtgaatagctgatgggaactagagaagatgctcagtagacagttattgtggagactatattactgattacccctgtttctgagtggttaggacaatgtgacaattgattttgggtattatttgtagatgtttttctttttgttaaaagtgccaagataggtgtgcagttgctgattctcagtttgctaagaattagctgtgtctgtatttcgtacctcagttgattctaagtgaacatttctttgaattgatgctttgttcttgcatcatgcaacttggtgaagctttcttgtagttgctccagtggcaatctagtctggtatgtttagaactcttgtgatggtatgagttcatcaagatattggtgatccaattagcctaaccaatgttttttaccccctattgtcactgacttatactcccttatctataaaaataattgtgacattgatccatctcctcacaatcattaatattatatgtactgaccatctttacactctcaacactgaatctaagtaggggaattttgggaaattcaatgatgaactagtacacccttcttcccaataatattgttgacctttttattttgatttgtcccatattgtcctctttggtaatttaatgtatattcacccaattttcttttcaatacccactataccaacatataattggttaattcatttttattaattatatttcctaagagcttgttgtgtaaacgtggatgaatttgtaggcatggatgaagtattgttataatgaggtgacaacattacttaatttcgaactgagggacagagggatatgatgataaaacaacttttgcttgcttcttaaactcagaagatagggtttacaccaagtggcatgtaaaagtcactagatgattatctattacaagggcttgtacaatctgaagtacgataggatttgaagttaacaacattcatcgaaagctcataacttgtccttatatcaatataagttgctggcatgtgaaattgcgttgcaagcatccatgagctagctcaactattaactattaaactttatatttttgcttgatctagtatgagtcctactatttagtttctccatctaccttaatatgtcgcatacaccaactaatcattatcgctagaatcaataaacaaagctttctttccttaggtgtattagtacctagctcctgtaataccaagagcacccaaattgggaagaaaaagtagaattggctcatatctctaatcctacattgatcattgaaaaggaccttaaggttctcatactgaaacatcatctttttgagcaggatatctacgtagacgacaagaaagactactttggttgcccgtgcatttgagtgcatcagacaacttctttaccactgtctaacggcttgctttggccatattgtggtcttctatgccaaaattaatgatatttcttggcaccgcgctaatgatattactgaatgcggatatcgtacgattagaatttattcaaagtaggtagcaattactagttttgagcattgagtttcaataattagtaaattaagtgctaaacttgtacattttggctacatgtatttgaattagaattggtacgaggaaatatagcaacattacgggcaatgttcactcaagtagaagccattacatcaaatagtactagttgaagtattagttctcataatactaatcattgtcattaatggaatattggaacgtaaatgcctttaaggtgctgtagttttagtagaaattctactattctagtatgataatgcaatttattgaaactgtttgtaagatagcttggatcccacatcagtcttgatgctaaataaatggatgtccataatcttctaatctttaatttgtgtctcttaccaaacgagaaaaaataggagaaatccaatttgcatgacctcaataaggaaatgttgttaatgtgtgatgcttgtttctcatttatagtctagagagagttatcatgtccaagattgcagtcttggtactgagaaagtttgattgttggttggctgcttcttgagcctcttttttttagagtaagacacttcctagatataattttctttatttttttgtaaattccatatatactactacattaacaggtttaagtttatattaggtgagagagattactcaccagtttgctccttatgttggtcgttggcaagctgaagctctgatggcccttcaagaggtgcagaccaactcttttagcctttttttttctggcatgtcaagtgtggctattagattttctgtgtgattctcactcccatatatctatatatgtacatattaaagcacattgatacctatcttgtcagatgtggtcttttcaattcttttctaagttgagattcttctcttggtcgtagatatgctcctgccgaaatatactgctgtcttgttatccatcatgacttggttatgcttgtatctgggcattatcttggcatgcttaaaaacaagtattgaacgagcctcctattgataaattttactattaatattggatggcttctcaaattctaatggcagtgagatactgttaagttgggagaaatagattaagaaacagaaagatgtttaccatgagagcaattgaaatagaaaatagagtaactttttgcaaagattttggtcctttagattgttgaatactacctgataatgaagcattttctaaatttatgtgctttctatctatcagatactggaatacaatcaaattcctatcacgtactgagcattgtgatcagattcttgcttgcttcctatcacatactggaatccttttgattgttgaatacaaagataatgaagcattctctaactttatgtgctgtaactacttataatgattcttgcttgcctcctatcacgtactcaaatcctttgtttgatttgtctcttataagaggaacttcctgtctttctttgtcatgacttagtatttatagaggtgccaacttatggccttgacaactgaagcttttatgcaaactccggattttgttgatggaagtacaagtaacactttagcatgtggattcaggtctaacggttaagactttttaatgaatgttttaactgtagtagtttattgatataaaaaaagtggtctctcaaactttttatgagatcatatcgaagtaatcaaatttatgattcaggtgcttctgctattattcttggttaagcatgtgctatttttgacagtctgtcaattgtaggctgcagagaattttattgtccgtttgtttgaagatggtatgctttgtgcaattcatgccaaacgagttacactcagtgagtatctgatttccttcggtggtgctgctattatgcattatatacactttgcctcaatatcgttatataaggagtccttgttttcatatttgtttgatgcatatgttatatcctgtttagtggctgctgcagttgtgaacttacggcctgtttgattagtggtcataaatgatggtaatactaatataatttagtataaatttgtaaaaaaaatgctaatatcaatatttatggtaatgaaattttatcataaaacatgagttctcttttataagttttcattactatccaataccaccttcccaagtggtaatgaacggtaatgaaattttaggaagaaaatggatatttggggattagatagcattaccatgggtaatgacatgagattttctttacaactttatactacgatgcattatcattaccaccatttatgacccataaccaaaaaaaccataatgtgttaggttcatttttcatttttctaataatttgcttcatgaattttttctggagatatcttatctagatatttcttgccaacatgtttcacctgataattgatcgatttaatagttcagaactttccaaaaactatgctgctcggtgttggctgtcatccatcagtttaagaaaactattgacatgatttaagcctcgtcctgtactactaggaagggtaaactattgttgcttccaaaaatgtcttttaagggcgtgttcagcaacaatagttgtagtagtagcttttagctgttagttgtgctcgtagctgttagtggttagtgtgtaactgttagctgttcaagtagcggtataagatattgatgttcggtaaaagaagctgtcaaaatagctgtttacaaagaattaataaaaaactcaaacaaagctttaatatataatttatgcaccactaaagctaccccaaaagctacaaattgtagctttttacaaacactactaaaacactacttgtaacactaaaagctacttatactactattttgccaaacattattattttttcttaattagtgttttgacctagtcaagacactaaaagctacttgaaaagcttttgccgaacacgcccttagtagacaagaggggggagggggtcatcaagaaaatatgattatactctcaacaaaaaaaaaatgtaacttaaaaaaaataaaaataaataattgactacttcaattaagaaaagaatagaataaaaacattacagtggatgtctcatccacatccctaatttaatggcacaatagaataattgttttaaattttagaaattacaacacaagatgtaaattactcttatcttcctcttcgtaatctttttactcttcctttacctcttcctttacctctacataaaatagagaattagagattgattaagataattataagattttagaaacattggttaagaaattcttcaacaaacataatcaagtaactccattattttagtttagtgacttgctatttatcaccctaatttcaccatctaccgccctccttggacaatattgccccttccactttcttcactcttccttcctcacgcatcttatcatctccttccactatcacctttaaaaaagtgtgtcaggcacaacaaaaacgcttttatcaacccacgcgaggcgaagtacgtcaggcgcaacaaggcgcgcacctaattctgtcttttgccaaggctgatggtgcacttagttttaaaaagcgcagcaaagatgtgcctaggcgcaaggcggtgaaaaaattgcatccgtcagcagcggagtagaggctcacaacaataggtgcgaagaggcgtgcacgtacaaaagaagcaaaaataagaaactcaaatatgagacccagtgtttaacatgtaaattcgatacccagtgtttaacatgtaaattcgattaaaagcccttaattaattgcatgaaattaattcattttaacctatactaaaagccctaatattagaaaatcctagtttgcaggttgaggaatttggaaaattgatgattgttggatttgaaaaaattgttgccggcgatgaatgtgaggtggtttatggcactagagaggttggcgttcgttgccgatgaagctttccaaggtcattctctccttgtcttcttcctatgcctagctctcttccctctccttaatcttctcttcttttctattctctctctttatcactacattatgtttatttctcgttcttcccctatgtctttcacttggacacttcgggggtatcttcatcttttatctgcaatttgaagtttgagaagcttccagagtcgagtgttaaacttttgcttctttttttttaatcttttgcccttttttcttagtggcccttgactagtgatgcacatgtgaccaattactaaatgagcttttattttgtctctcttctttttcaagcaattttttttaagtaaatcatctaaaacaaagtactatccattttagttgtgtaaatggtgctattttaaaaccgcacaaaaattaaaaacataaaaataaaggtgtgcttcgcatacaagatgtatgcgccttcgtcttgccccttttgagactaagactaccataagaacttagtcacttgagaatggaatgggtgcaagatggacgacgataattctaaagacctctagaaggatagtgtatagtaactaatacgaaccgaaatataagtttaactaaaattttaaagtctatatttccatatggtatatgctggaatacacgaaatgtccagaatttgtagtggaccacgatccacacgtcttttcaggattctaggtgtattccaacgaaaaatataagaaaaccatattctactatctggttgttgtcatcctttccttgccggcgtgacttctcatccttttatttttgtccggtgctggtgacacactttcctatgatagtgtggtgcaaagtaaggtgatgatatggtgttttgtagaggtgtggtgatttttgtggtggtgggtggaagaggggtggttgcatatagaaaggggtaagagtcaatgaggggtggaaggggacaaggggtatattggtaaatgcatgtaacattagggtggtgttgagtaatttttgggaagttaatataaactacccccttttggtacaagagagaatacccgaactactgctctgatatttttgttcacgttatttgatgtaattacgcaattaatttgttttctataagcttccgcacacaattgtgcatataaggctagtctaatatgagacaccaacataactgactttcttttgcaacgaaggtaccttgtcagatttagaacatagcatcaggattttatttgttgtatctgtcatccttgtttattgctttaattatgctttgtatgatgcattttaccacttcgtatgaaaaaaagtgaaatttcatttagtggtcatttacatattacgagttgtggacatgtttgaacatttgattttggaaattttaagcctcatattatggagatttattggacacaaatatagccataattctccatcaacttgtttctagaagtgttgctcttcctgatgtacttgaattctaattaggttttatcagacattatattataatgatatgatttacaatttgttgtagtgaaaaaggatttggagctcgcgcgaaggattgggggcagagagaggggatggtaactaaacaacacagatgactcatttatttaagggccaacaattgaattcgctgttgatttcatctgtatatactgctctaggcttctattccaatgtaatttataaatccaaggttagtagcatgttaagctttgtattcagtataatgagacttatattttgcagttgagattttagttgtttgatgtgacttgtaaattgtaacttgtaagtgacgtcttgaggattatcgggacaatatactattttttttttcaaa

SEQ ID NO: 22 - DNA, 462 bp, Artificial Sequence
  Sorghum bicolor - cDNA coding for CENH3
atgagagttaaacacactgctgccaggaaatcaaccaccaatggtcctcgttcaaaggctcagaaatctccgcgcagtttgcaatcaccacaatcgccttctagtagttcaaagcgcaaatcacgcagaaacactgatgcaactcctcaaaagaagaaggcttaccgccgtaagccgggcactgtggcactctgggaaatacgcaaatttcagaagtcattcaagcccttgattcctgctgcgcctttcattcgaacagtgagagagattactcaccagtttgctccttatgttggtcgttggcaagctgaagctctgatggcccttcaagaggctgcagagaattttattgtccgtttgtttgaagatggtatgctttgtgcaattcatgccaaacgagttacactcatgaaaaaggatttggagctcgcgcgaaggattgggggcagagagaggggatgg

SEQ ID NO: 23 - protein, 154 aa, Beta vulgaris
MRVKHTAARKSTTNGPRSKAQKSPRSLQSPQSPSSSSKRKSRRNTDATPQKKKAYRRKPGTVALWEIRKFQKSFKPLIPAAPFIRTVREITHQFAPYVGRWQAEALMALQEAAENFIVRLFEDGMLCAIHAKRVTLMKKDLELARRIGGRERGW

SEQ ID NO: 24 - DNA, 4597 bp, Artificial Sequence
  Z. mays CENH3-Mu-mutation
  misc_recomb (676)..(685): transposon insertion
agagacggaaagagtatatatatttgttttgctattatttaaagtattaaaagatagtggacgaatgaacgtcctctatgtttaaaagaacgttttagaggacgttgtgttgttgaaggaaatatgaaaaaaaaatcttctgcatatttagaagggaggagcgtttacacattactttcgggacttcaacccaaatatgtcaaggtttgtgagtggctcagtgcggaaaaaaaatcctatatataccagatgtaaacactatcttttacagcctatcacattcacatttagaggttcacaaagatagatcaaaatttataaaataatcatttaatattttttttattttatttatatggataagcagctggtgtatgtgaggagctgtaaaagatattttttacatccgagatgtaaagattttttttaactcaatgctggttaccggctgggaggacgatgataaagaaagcatctctcactgcattccgggcccactactcaaacgttcggcacgccaggttggcaggtagccgttacatcgataggcactcggccactcgcacgcagacaccacaccagtgtgctcagtgctcactgctcaccataataacgctgcacctcttttcatttcaccatctcctgcccccttaaaaaaaagactcaccgtcgacacgccctcccgtcccgagagttctgaatcgaaaccgtcggccacgagagcagtgcgaggcgcccaccgcgatggctcgaaccaagcaccaggccgtgaggaagacggcggagaagcccaagaagaagctccagttcgagcgctcaggtaacccgggtcccgcgctcccccccgcttcgcaagcagacgctgtcgcttctctccgaccctggtgctaagcacgttccttgttccgtcttttgcaggtggtgcgagtacctcggcgacgccggtgagcgcgtgcgtgcggggatcagttccctccttttgcctttttttgttgggctgctcttacttgcttgcaagctgtttgatggaatgcaggaaagggctgctgggaccgggggaagagcggcgtctggaggtgactcaggtgaggacctatttgtcgttgctggatgctgggtttcgcttgcaatctaattttgttgcaagatgagggcgaatgtgccagttccatgtgggtgtcatggtctcggagttactaccttaattgctcaccatagtatgttttcttaaaaaaaacagttaagaagacgaaaccacgccaccgctggcggccagggactgtagcgctgcgggagatcaggaagtaccagaagtccactgaaccgctcatcccctttgcgcctttcgtccgtgtggtgggtgcaggcgtgtttgtcctctgcatagtatggggttgttccgcattctgtctaatggaaagttattcttctgagaaaaaaaatgcaggtgagggagttaaccaatttcgtaacaaacgggaaagtagagcgctataccgcagaagccctccttgcgctgcaagaggtcagttatgaaaaatgtcttatctctctgttaagatcctcttcatatacatagttgctattgctatcgtgaagtcttttttttctgttaattggtctggtactacttactagtcaggatttcatattgcggtttttcctagtggtgtgtagttaaaaagtagtttaattgcttttagttaaaaggggtgttcagggctaaagatcaactatgagaaaacagaaattttcccaattcgatacccgacagcattatggcctgcgctaatggaggtgtttccgggcaaatactctagcctacctgggaagtaccttgggttgccccttcatttcaggaaagtaaaaaggaatgatcttcaacctctaatcgaaaaaatcaacaacaggctggccttgctggaaaggcaagatgttgtccaaggctggtatagaaactcttgtaaaatcgatgctatccgcacaaccaatctaccatctaatggtttttccacctcaaaaatggctgctgcaaacaattgacaaaatacgaagaaacttcctgtggagagggagcaatccagaagtttgcagcgggggtcactgcctcgtcaactggcccgtaacttgcctcccaaagaacaagggaggtcttggaattctggaccttgatcgttttgcgagggggctaagactaagatggctgtggctacgatggaagagcaaagatagggcgtggactgccttgaagcttccttgtgacaaaactgatgaagatctcttcaatgcttccacaactgtcacggtaggcaatggaaagatagctgaattctggaattctagttggatccaaggccaagcccctaagaacattgcgccaacactgttcaagaaggaaaagaggaagaacatcacggtcgccaaagcgctcactaacaacaattggattcgtttatgctcaccatacacgggtgagggggagtttagagaggtcgtctctctttggcaggccataggtaacatgcaagagcttaacggtttggaagacaacatctcttggagatggacggcagatgggcagtacagtgctagcagtgcatacaaaatccagttcgcatccaatttcactaaaatgaacctctgccctatttggaaggctaaagtggaaccgaaatgccgattttttgcttggacactacttcataagagaattctgactgccgataaccttcataaaagaggttgcaactcagcctcagaaacaattccccacttatgcaaggattgcccctttagtagagaggtgtggaacaaagttttgtctcgggccaactttcctttactgactgggtctcccagtgacacttctttgtatgattggtggacggacatgtgcagcctttgcagcagacaggcaagaagaggtttcgacggtctgctatttcacttttggtggaacttatggctggaaagaaataacagaatctttcaaaggcagcgtagaagtgtagatcaagttgctctggcagtcaaggattatgctagtagctgaagtctagttggtttggactagtggttttgttgcttttctttttaatttctttttagttctttttatgttgttttcgtttccttaagttgcttggagtctgtattatcctctttcttctaatatagatcggagcgacaaaccttttgccccttcctttcaaaaaaaagttaaaagggaatttaactgctttcctagtggtgtagttaaaatggatttcatattgcggcctttcctagcttgcttgctattgattggactatagtgatccaaatgctgataactttgtcgcttgtgtaggcatggttagagagcttagagtttgcatttattcaataccttgagactgcatttcatatacataaattattcatgattatttcttttctctatttgttctggttaattaagagttttaggtttccatatttttgtacgtgcatcatttaaattcttgtattgtttttcgttcttgtctacaggcagcagaattccacttgatagaactgtttgaaatggcgaatctgtgtgccatccatgccaagcgtgtcacaatcagtaagttatcactgagtgaactcctttttctctgtagcattactcctaatgaatatgtgtgatgcattttggttgcacgattctttagtgattctgcttcagatggatatgataaatctagatgttattttgaagtggcgaattgcttacgagcggaaatagtaatgttcaaatagcgcaaagtgcaactgttgacttttagtaggccatttatatggtttgattaccaacaaatacgtcaatcatatgatttgattatcaacaaaggaatcagctatatggtttgattatcaacaaaggaatcagctaggtttgcttatcaacattcaacaaaggcatcaagtaatactccatccgtttcaatttataattcgtttgactttttttatctaagtttgatcggctcgacttattaaaaaaaatcataattattgttaatttttgttgtgatattgtttagtataatatactttaaatgtgactttgagtttttcattttttcgcaaaaaaaaatgaataggacgagccggtcaaacgtgacacaaaaaagtcaaacgaattataatttgggacacacggagtagtaaataatgtaacaacttagagagtgggacaaaaaaatctctagtggtgctaaatttagttcagctttgtataaacacaagcattgattgagaaatctgacaactcaaggatctgtaggaaatgtgttaccctaaatgttttccttactgatgcagtgcaaaaggacatacaacttgcaaggcgtatcggaggaaggcgttgggcatgatatataatatccattctgattgcatcattcttgtgaatttgtttgtaggagctagacattagtgttgttgaatgctgcatggttcctaatccttttcgcagtctaacatctgtggagttagtatgttacatggcaacagctgaacatctgtggactatatggcaacagccgaagattgtgtctgtgggataactggt